European Patent Specification EP 3 652 203 B1, published July 2, 2025. Title: Engineered TSC2. Applicant: The John Hopkins University. The sequence listing filed with the application follows.

SEQUENCE LISTING (11 sequences)

SEQ ID NO: 1 - protein, 1807 aa, Artificial Sequence
  human TSC2 polypeptide having a S1364A substitution
MAKPTSKDSGLKEKFKILLGLGTPRPNPRSAEGKQTEFIITAEILRELSMECGLNNRIRMIGQICEVAKTKKFEEHAVEALWKAVADLLQPERPLEARHAVLALLKAIVQGQGERLGVLRALFFKVIKDYPSNEDLHERLEVFKALTDNGRHITYLEEELADFVLQWMDVGLSSEFLLVLVNLVKFNSCYLDEYIARMVQMICLLCVRTASSVDIEVSLQVLDAVVCYNCLPAESLPLFIVTLCRTINVKELCEPCWKLMRNLLGTHLGHSAIYNMCHLMEDRAYMEDAPLLRGAVFFVGMALWGAHRLYSLRNSPTSVLPSFYQAMACPNEVVSYEIVLSITRLIKKYRKELQVVAWDILLNIIERLLQQLQTLDSPELRTIVHDLLTTVEELCDQNEFHGSQERYFELVERCADQRPESSLLNLISYRAQSIHPAKDGWIQNLQALMERFFRSESRGAVRIKVLDVLSFVLLINRQFYEEELINSVVISQLSHIPEDKDHQVRKLATQLLVDLAEGCHTHHFNSLLDIIEKVMARSLSPPPELEERDVAAYSASLEDVKTAVLGLLVILQTKLYTLPASHATRVYEMLVSHIQLHYKHSYTLPIASSIRLQAFDFLLLLRADSLHRLGLPNKDGVVRFSPYCVCDYMEPERGSEKKTSGPLSPPTGPPGPAPAGPAVRLGSVPYSLLFRVLLQCLKQESDWKVLKLVLGRLPESLRYKVLIFTSPCSVDQLCSALCSMLSGPKTLERLRGAPEGFSRTDLHLAVVPVLTALISYHNYLDKTKQREMVYCLEQGLIHRCASQCVVALSICSVEMPDIIIKALPVLVVKLTHISATASMAVPLLEFLSTLARLPHLYRNFAAEQYASVFAISLPYTNPSKFNQYIVCLAHHVIAMWFIRCRLPFRKDFVPFITKGLRSNVLLSFDDTPEKDSFRARSTSLNERPKSLRIARPPKQGLNNSPPVKEFKESSAAEAFRCRSISVSEHVVRSRIQTSLTSASLGSADENSVAQADDSLKNLHLELTETCLDMMARYVFSNFTAVPKRSPVGEFLLAGGRTKTWLVGNKLVTVTTSVGTGTRSLLGLDSGELQSGPESSSSPGVHVRQTKEAPAKLESQAGQQVSRGARDRVRSMSGGHGLRVGALDVPASQFLGSATSPGPRTAPAAKPEKASAGTRVPVQEKTNLAAYVPLLTQGWAEILVRRPTGNTSWLMSLENPLSPFSSDINNMPLQELSNALMAAERFKEHRDTALYKSLSVPAASTAKPPPLPRSNTVASFSSLYQSSCQGQLHRSVSWADSAVVMEEGSPGEVPVLVEPPGLEDVEAALGMDRRTDAYSRSSSVSSQEEKSLHAEELVGRGIPIERVVASEGGRPSVDLSFQPSQPLSKSSSSPELQTLQDILGDPGDKADVGRLSPEVKARSQSGTLDGESAAWSASGEDSRGQPEGPLPSSSPRSPSGLRPRGYTISDSAPSRRGKRVERDALKSRATASNAEKVPGINPSFVFLQLYHSPFFGDESNKPILLPNESQSFERSVQLLDQIPSYDTHKIAVLYVGEGQSNSELAILSNEHGSYRYTEFLTGLGRLIELKDCQPDKVYLGGLDVCGEDGQFTYCWHDDIMQAVFHIATLMPTKDVDKHRCDKKRHLGNDFVSIVYNDSGEDFKLGTIKGQFNFVHVIVTPLDYECNLVSLQCRKDMEGLVDTSVAKIVSDRNLPFVARQMALHANMASQVHHSRSNPTDIYPSKWIARLRHIKRLRQRICEEAAYSNPSLPLVHPPSHSKAPAQTPAEPTPGYEVGQRKRLISSVEDFTEFV

SEQ ID NO: 2 - protein, 1807 aa, Artificial Sequence
  human TSC2 polypeptide having a S1364E substitution
MAKPTSKDSGLKEKFKILLGLGTPRPNPRSAEGKQTEFIITAEILRELSMECGLNNRIRMIGQICEVAKTKKFEEHAVEALWKAVADLLQPERPLEARHAVLALLKAIVQGQGERLGVLRALFFKVIKDYPSNEDLHERLEVFKALTDNGRHITYLEEELADFVLQWMDVGLSSEFLLVLVNLVKFNSCYLDEYIARMVQMICLLCVRTASSVDIEVSLQVLDAVVCYNCLPAESLPLFIVTLCRTINVKELCEPCWKLMRNLLGTHLGHSAIYNMCHLMEDRAYMEDAPLLRGAVFFVGMALWGAHRLYSLRNSPTSVLPSFYQAMACPNEVVSYEIVLSITRLIKKYRKELQVVAWDILLNIIERLLQQLQTLDSPELRTIVHDLLTTVEELCDQNEFHGSQERYFELVERCADQRPESSLLNLISYRAQSIHPAKDGWIQNLQALMERFFRSESRGAVRIKVLDVLSFVLLINRQFYEEELINSVVISQLSHIPEDKDHQVRKLATQLLVDLAEGCHTHHFNSLLDIIEKVMARSLSPPPELEERDVAAYSASLEDVKTAVLGLLVILQTKLYTLPASHATRVYEMLVSHIQLHYKHSYTLPIASSIRLQAFDFLLLLRADSLHRLGLPNKDGVVRFSPYCVCDYMEPERGSEKKTSGPLSPPTGPPGPAPAGPAVRLGSVPYSLLFRVLLQCLKQESDWKVLKLVLGRLPESLRYKVLIFTSPCSVDQLCSALCSMLSGPKTLERLRGAPEGFSRTDLHLAVVPVLTALISYHNYLDKTKQREMVYCLEQGLIHRCASQCVVALSICSVEMPDIIIKALPVLVVKLTHISATASMAVPLLEFLSTLARLPHLYRNFAAEQYASVFAISLPYTNPSKFNQYIVCLAHHVIAMWFIRCRLPFRKDFVPFITKGLRSNVLLSFDDTPEKDSFRARSTSLNERPKSLRIARPPKQGLNNSPPVKEFKESSAAEAFRCRSISVSEHVVRSRIQTSLTSASLGSADENSVAQADDSLKNLHLELTETCLDMMARYVFSNFTAVPKRSPVGEFLLAGGRTKTWLVGNKLVTVTTSVGTGTRSLLGLDSGELQSGPESSSSPGVHVRQTKEAPAKLESQAGQQVSRGARDRVRSMSGGHGLRVGALDVPASQFLGSATSPGPRTAPAAKPEKASAGTRVPVQEKTNLAAYVPLLTQGWAEILVRRPTGNTSWLMSLENPLSPFSSDINNMPLQELSNALMAAERFKEHRDTALYKSLSVPAASTAKPPPLPRSNTVASFSSLYQSSCQGQLHRSVSWADSAVVMEEGSPGEVPVLVEPPGLEDVEAALGMDRRTDAYSRSSSVSSQEEKSLHAEELVGRGIPIERVVESEGGRPSVDLSFQPSQPLSKSSSSPELQTLQDILGDPGDKADVGRLSPEVKARSQSGTLDGESAAWSASGEDSRGQPEGPLPSSSPRSPSGLRPRGYTISDSAPSRRGKRVERDALKSRATASNAEKVPGINPSFVFLQLYHSPFFGDESNKPILLPNESQSFERSVQLLDQIPSYDTHKIAVLYVGEGQSNSELAILSNEHGSYRYTEFLTGLGRLIELKDCQPDKVYLGGLDVCGEDGQFTYCWHDDIMQAVFHIATLMPTKDVDKHRCDKKRHLGNDFVSIVYNDSGEDFKLGTIKGQFNFVHVIVTPLDYECNLVSLQCRKDMEGLVDTSVAKIVSDRNLPFVARQMALHANMASQVHHSRSNPTDIYPSKWIARLRHIKRLRQRICEEAAYSNPSLPLVHPPSHSKAPAQTPAEPTPGYEVGQRKRLISSVEDFTEFV

SEQ ID NO: 3 - DNA, 5424 bp, Artificial Sequence
  nucleic acid encoding a human TSC2 polypeptide having a S1364A substitution
atggccaaaccaacaagcaaagattcaggcttgaaggagaagtttaagattctgttgggactgggaacaccgaggccaaatcccaggtctgcagagggtaaacagacggagtttatcatcaccgcggaaatactgagagaactgagcatggaatgtggcctcaacaatcgcatccggatgatagggcagatttgtgaagtcgcaaaaaccaagaaatttgaagagcacgcagtggaagcactctggaaggcggtcgcggatctgttgcagccggagcggccgctggaggcccggcacgcggtgctggctctgctgaaggccatcgtgcaggggcagggcgagcgtttgggggtcctcagagccctcttctttaaggtcatcaaggattacccttccaacgaagaccttcacgaaaggctggaggttttcaaggccctcacagacaatgggagacacatcacctacttggaggaagagctggctgactttgtcctgcagtggatggatgttggcttgtcctcggaattccttctggtgctggtgaacttggtcaaattcaatagctgttacctcgacgagtacatcgcaaggatggttcagatgatctgtctgctgtgcgtccggaccgcgtcctctgtggacatagaggtctccctgcaggtgctggacgccgtggtctgctacaactgcctgccggctgagagcctcccgctgttcatcgttaccctctgtcgcaccatcaacgtcaaggagctctgcgagccttgctggaagctgatgcggaacctccttggcacccacctgggccacagcgccatctacaacatgtgccacctcatggaggacagagcctacatggaggacgcgcccctgctgagaggagccgtgttttttgtgggcatggctctctggggagcccaccggctctattctctcaggaactcgccgacatctgtgttgccatcattttaccaggccatggcatgtccgaacgaggtggtgtcctatgagatcgtcctgtccatcaccaggctcatcaagaagtataggaaggagctccaggtggtggcgtgggacattctgctgaacatcatcgaacggctccttcagcagctccagaccttggacagcccggagctcaggaccatcgtccatgacctgttgaccacggtggaggagctgtgtgaccagaacgagttccacgggtctcaggagagatactttgaactggtggagagatgtgcggaccagaggcctgagtcctccctcctgaacctgatctcctatagagcgcagtccatccacccggccaaggacggctggattcagaacctgcaggcgctgatggagagattcttcaggagcgagtcccgaggcgccgtgcgcatcaaggtgctggacgtgctgtcctttgtgctgctcatcaacaggcagttctatgaggaggagctgattaactcagtggtcatctcgcagctctcccacatccccgaggataaagaccaccaggtccgaaagctggccacccagttgctggtggacctggcagagggctgccacacacaccacttcaacagcctgctggacatcatcgagaaggtgatggcccgctccctctccccacccccggagctggaagaaagggatgtggccgcatactcggcctccttggaggatgtgaagacagccgtcctggggcttctggtcatccttcagaccaagctgtacaccctgcctgcaagccacgccacgcgtgtgtatgagatgctggtcagccacattcagctccactacaagcacagctacaccctgccaatcgcgagcagcatccggctgcaggcctttgacttcctgttgctgctgcgggccgactcactgcaccgcctgggcctgcccaacaaggatggagtcgtgcggttcagcccctactgcgtctgcgactacatggagccagagagaggctctgagaagaagaccagcggccccctttctcctcccacagggcctcctggcccggcgcctgcaggccccgccgtgcggctggggtccgtgccctactccctgctcttccgcgtcctgctgcagtgcttgaagcaggagtctgactggaaggtgctgaagctggttctgggcaggctgcctgagtccctgcgctataaagtgctcatctttacttccccttgcagtgtggaccagctgtgctctgctctctgctccatgctttcaggcccaaagacactggagcggctccgaggcgccccagaaggcttctccagaactgacttgcacctggccgtggttccagtgctgacagcattaatctcttaccataactacctggacaaaaccaaacagcgcgagatggtctactgcctggagcagggcctcatccaccgctgtgccagccagtgcgtcgtggccttgtccatctgcagcgtggagatgcctgacatcatcatcaaggcgctgcctgttctggtggtgaagctcacgcacatctcagccacagccagcatggccgtcccactgctggagttcctgtccactctggccaggctgccgcacctctacaggaactttgccgcggagcagtatgccagtgtgttcgccatctccctgccgtacaccaacccctccaagtttaatcagtacatcgtgtgtctggcccatcacgtcatagccatgtggttcatcaggtgccgcctgcccttccggaaggattttgtccctttcatcactaagggcctgcggtccaatgtcctcttgtcttttgatgacacccccgagaaggacagcttcagggcccggagtactagtctcaacgagagacccaagagtctgaggatagccagaccccccaaacaaggcttgaataactctccacccgtgaaagaattcaaggagagctctgcagccgaggccttccggtgccgcagcatcagtgtgtctgaacatgtggtccgcagcaggatacagacgtccctcaccagtgccagcttggggtctgcagatgagaactccgtggcccaggctgacgatagcctgaaaaacctccacctggagctcacggaaacctgtctggacatgatggctcgatacgtcttctccaacttcacggctgtcccgaagaggtctcctgtgggcgagttcctcctagcgggtggcaggaccaaaacctggctggttgggaacaagcttgtcactgtgacgacaagcgtgggaaccgggacccggtcgttactaggcctggactcgggggagctgcagtccggcccggagtcgagctccagccccggggtgcatgtgagacagaccaaggaggcgccggccaagctggagtcccaggctgggcagcaggtgtcccgtggggcccgggatcgggtccgttccatgtcggggggccatggtcttcgagttggcgccctggacgtgccggcctcccagttcctgggcagtgccacttctccaggaccacggactgcaccagccgcgaaacctgagaaggcctcagctggcacccgggttcctgtgcaggagaagacgaacctggcggcctatgtgcccctgctgacccagggctgggcggagatcctggtccggaggcccacagggaacaccagctggctgatgagcctggagaacccgctcagccctttctcctcggacatcaacaacatgcccctgcaggagctgtctaacgccctcatggcggctgagcgcttcaaggagcaccgggacacagccctgtacaagtcactgtcggtgccggcagccagcacggccaaaccccctcctctgcctcgctccaacacagtggcctctttctcctccctgtaccagtccagctgccaaggacagctgcacaggagcgtttcctgggcagactccgccgtggtcatggaggagggaagtccgggcgaggttcctgtgctggtggagcccccagggttggaggacgttgaggcagcgctaggcatggacaggcgcacggatgcctacagcaggtcgtcctcagtctccagccaggaggagaagtcgctccacgcggaggagctggttggcaggggcatccccatcgagcgagtcgtcgcctcggagggtggccggccctctgtggacctctccttccagccctcgcagcccctgagcaagtccagctcctctcccgagctgcagactctgcaggacatcctcggggaccctggggacaaggccgacgtgggccggctgagccctgaggttaaggcccggtcacagtcagggaccctggacggggaaagtgctgcctggtcggcctcgggcgaagacagtcggggccagcccgagggtcccttgccttccagctccccccgctcgcccagtggcctccggccccgaggttacaccatctccgactcggccccatcacgcaggggcaagagagtagagagggacgccttaaagagcagagccacagcctccaatgcagagaaagtgccaggcatcaaccccagtttcgtgttcctgcagctctaccattcccccttctttggcgacgagtcaaacaagccaatcctgctgcccaatgagtcacagtcctttgagcggtcggtgcagctcctcgaccagatcccatcatacgacacccacaagatcgccgtcctgtatgttggagaaggccagagcaacagcgagctcgccatcctgtccaatgagcatggctcctacaggtacacggagttcctgacgggcctgggccggctcatcgagctgaaggactgccagccggacaaggtgtacctgggaggcctggacgtgtgtggtgaggacggccagttcacctactgctggcacgatgacatcatgcaagccgtcttccacatcgccaccctgatgcccaccaaggacgtggacaagcaccgctgcgacaagaagcgccacctgggcaacgactttgtgtccattgtctacaatgactccggtgaggacttcaagcttggcaccatcaagggccagttcaactttgtccacgtgatcgtcaccccgctggactacgagtgcaacctggtgtccctgcagtgcaggaaagacatggagggccttgtggacaccagcgtggccaagatcgtgtctgaccgcaacctgcccttcgtggcccgccagatggccctgcacgcaaatatggcctcacaggtgcatcatagccgctccaaccccaccgatatctacccctccaagtggattgcccggctccgccacatcaagcggctccgccagcggatctgcgaggaagccgcctactccaaccccagcctacctctggtgcaccctccgtcccatagcaaagcccctgcacagactccagccgagcccacacctggctatgaggtgggccagcggaagcgcctcatctcctcggtggaggacttcaccgagtttgtgtga

SEQ ID NO: 4 - DNA, 5424 bp, Artificial Sequence
  nucleic acid encoding a human TSC2 polypeptide having a S1364E substitution
atggccaaaccaacaagcaaagattcaggcttgaaggagaagtttaagattctgttgggactgggaacaccgaggccaaatcccaggtctgcagagggtaaacagacggagtttatcatcaccgcggaaatactgagagaactgagcatggaatgtggcctcaacaatcgcatccggatgatagggcagatttgtgaagtcgcaaaaaccaagaaatttgaagagcacgcagtggaagcactctggaaggcggtcgcggatctgttgcagccggagcggccgctggaggcccggcacgcggtgctggctctgctgaaggccatcgtgcaggggcagggcgagcgtttgggggtcctcagagccctcttctttaaggtcatcaaggattacccttccaacgaagaccttcacgaaaggctggaggttttcaaggccctcacagacaatgggagacacatcacctacttggaggaagagctggctgactttgtcctgcagtggatggatgttggcttgtcctcggaattccttctggtgctggtgaacttggtcaaattcaatagctgttacctcgacgagtacatcgcaaggatggttcagatgatctgtctgctgtgcgtccggaccgcgtcctctgtggacatagaggtctccctgcaggtgctggacgccgtggtctgctacaactgcctgccggctgagagcctcccgctgttcatcgttaccctctgtcgcaccatcaacgtcaaggagctctgcgagccttgctggaagctgatgcggaacctccttggcacccacctgggccacagcgccatctacaacatgtgccacctcatggaggacagagcctacatggaggacgcgcccctgctgagaggagccgtgttttttgtgggcatggctctctggggagcccaccggctctattctctcaggaactcgccgacatctgtgttgccatcattttaccaggccatggcatgtccgaacgaggtggtgtcctatgagatcgtcctgtccatcaccaggctcatcaagaagtataggaaggagctccaggtggtggcgtgggacattctgctgaacatcatcgaacggctccttcagcagctccagaccttggacagcccggagctcaggaccatcgtccatgacctgttgaccacggtggaggagctgtgtgaccagaacgagttccacgggtctcaggagagatactttgaactggtggagagatgtgcggaccagaggcctgagtcctccctcctgaacctgatctcctatagagcgcagtccatccacccggccaaggacggctggattcagaacctgcaggcgctgatggagagattcttcaggagcgagtcccgaggcgccgtgcgcatcaaggtgctggacgtgctgtcctttgtgctgctcatcaacaggcagttctatgaggaggagctgattaactcagtggtcatctcgcagctctcccacatccccgaggataaagaccaccaggtccgaaagctggccacccagttgctggtggacctggcagagggctgccacacacaccacttcaacagcctgctggacatcatcgagaaggtgatggcccgctccctctccccacccccggagctggaagaaagggatgtggccgcatactcggcctccttggaggatgtgaagacagccgtcctggggcttctggtcatccttcagaccaagctgtacaccctgcctgcaagccacgccacgcgtgtgtatgagatgctggtcagccacattcagctccactacaagcacagctacaccctgccaatcgcgagcagcatccggctgcaggcctttgacttcctgttgctgctgcgggccgactcactgcaccgcctgggcctgcccaacaaggatggagtcgtgcggttcagcccctactgcgtctgcgactacatggagccagagagaggctctgagaagaagaccagcggccccctttctcctcccacagggcctcctggcccggcgcctgcaggccccgccgtgcggctggggtccgtgccctactccctgctcttccgcgtcctgctgcagtgcttgaagcaggagtctgactggaaggtgctgaagctggttctgggcaggctgcctgagtccctgcgctataaagtgctcatctttacttccccttgcagtgtggaccagctgtgctctgctctctgctccatgctttcaggcccaaagacactggagcggctccgaggcgccccagaaggcttctccagaactgacttgcacctggccgtggttccagtgctgacagcattaatctcttaccataactacctggacaaaaccaaacagcgcgagatggtctactgcctggagcagggcctcatccaccgctgtgccagccagtgcgtcgtggccttgtccatctgcagcgtggagatgcctgacatcatcatcaaggcgctgcctgttctggtggtgaagctcacgcacatctcagccacagccagcatggccgtcccactgctggagttcctgtccactctggccaggctgccgcacctctacaggaactttgccgcggagcagtatgccagtgtgttcgccatctccctgccgtacaccaacccctccaagtttaatcagtacatcgtgtgtctggcccatcacgtcatagccatgtggttcatcaggtgccgcctgcccttccggaaggattttgtccctttcatcactaagggcctgcggtccaatgtcctcttgtcttttgatgacacccccgagaaggacagcttcagggcccggagtactagtctcaacgagagacccaagagtctgaggatagccagaccccccaaacaaggcttgaataactctccacccgtgaaagaattcaaggagagctctgcagccgaggccttccggtgccgcagcatcagtgtgtctgaacatgtggtccgcagcaggatacagacgtccctcaccagtgccagcttggggtctgcagatgagaactccgtggcccaggctgacgatagcctgaaaaacctccacctggagctcacggaaacctgtctggacatgatggctcgatacgtcttctccaacttcacggctgtcccgaagaggtctcctgtgggcgagttcctcctagcgggtggcaggaccaaaacctggctggttgggaacaagcttgtcactgtgacgacaagcgtgggaaccgggacccggtcgttactaggcctggactcgggggagctgcagtccggcccggagtcgagctccagccccggggtgcatgtgagacagaccaaggaggcgccggccaagctggagtcccaggctgggcagcaggtgtcccgtggggcccgggatcgggtccgttccatgtcggggggccatggtcttcgagttggcgccctggacgtgccggcctcccagttcctgggcagtgccacttctccaggaccacggactgcaccagccgcgaaacctgagaaggcctcagctggcacccgggttcctgtgcaggagaagacgaacctggcggcctatgtgcccctgctgacccagggctgggcggagatcctggtccggaggcccacagggaacaccagctggctgatgagcctggagaacccgctcagccctttctcctcggacatcaacaacatgcccctgcaggagctgtctaacgccctcatggcggctgagcgcttcaaggagcaccgggacacagccctgtacaagtcactgtcggtgccggcagccagcacggccaaaccccctcctctgcctcgctccaacacagtggcctctttctcctccctgtaccagtccagctgccaaggacagctgcacaggagcgtttcctgggcagactccgccgtggtcatggaggagggaagtccgggcgaggttcctgtgctggtggagcccccagggttggaggacgttgaggcagcgctaggcatggacaggcgcacggatgcctacagcaggtcgtcctcagtctccagccaggaggagaagtcgctccacgcggaggagctggttggcaggggcatccccatcgagcgagtcgtcgagtcggagggtggccggccctctgtggacctctccttccagccctcgcagcccctgagcaagtccagctcctctcccgagctgcagactctgcaggacatcctcggggaccctggggacaaggccgacgtgggccggctgagccctgaggttaaggcccggtcacagtcagggaccctggacggggaaagtgctgcctggtcggcctcgggcgaagacagtcggggccagcccgagggtcccttgccttccagctccccccgctcgcccagtggcctccggccccgaggttacaccatctccgactcggccccatcacgcaggggcaagagagtagagagggacgccttaaagagcagagccacagcctccaatgcagagaaagtgccaggcatcaaccccagtttcgtgttcctgcagctctaccattcccccttctttggcgacgagtcaaacaagccaatcctgctgcccaatgagtcacagtcctttgagcggtcggtgcagctcctcgaccagatcccatcatacgacacccacaagatcgccgtcctgtatgttggagaaggccagagcaacagcgagctcgccatcctgtccaatgagcatggctcctacaggtacacggagttcctgacgggcctgggccggctcatcgagctgaaggactgccagccggacaaggtgtacctgggaggcctggacgtgtgtggtgaggacggccagttcacctactgctggcacgatgacatcatgcaagccgtcttccacatcgccaccctgatgcccaccaaggacgtggacaagcaccgctgcgacaagaagcgccacctgggcaacgactttgtgtccattgtctacaatgactccggtgaggacttcaagcttggcaccatcaagggccagttcaactttgtccacgtgatcgtcaccccgctggactacgagtgcaacctggtgtccctgcagtgcaggaaagacatggagggccttgtggacaccagcgtggccaagatcgtgtctgaccgcaacctgcccttcgtggcccgccagatggccctgcacgcaaatatggcctcacaggtgcatcatagccgctccaaccccaccgatatctacccctccaagtggattgcccggctccgccacatcaagcggctccgccagcggatctgcgaggaagccgcctactccaaccccagcctacctctggtgcaccctccgtcccatagcaaagcccctgcacagactccagccgagcccacacctggctatgaggtgggccagcggaagcgcctcatctcctcggtggaggacttcaccgagtttgtgtga

SEQ ID NO: 5 - protein, 1807 aa, Homo sapiens
MAKPTSKDSGLKEKFKILLGLGTPRPNPRSAEGKQTEFIITAEILRELSMECGLNNRIRMIGQICEVAKTKKFEEHAVEALWKAVADLLQPERPLEARHAVLALLKAIVQGQGERLGVLRALFFKVIKDYPSNEDLHERLEVFKALTDNGRHITYLEEELADFVLQWMDVGLSSEFLLVLVNLVKFNSCYLDEYIARMVQMICLLCVRTASSVDIEVSLQVLDAVVCYNCLPAESLPLFIVTLCRTINVKELCEPCWKLMRNLLGTHLGHSAIYNMCHLMEDRAYMEDAPLLRGAVFFVGMALWGAHRLYSLRNSPTSVLPSFYQAMACPNEVVSYEIVLSITRLIKKYRKELQVVAWDILLNIIERLLQQLQTLDSPELRTIVHDLLTTVEELCDQNEFHGSQERYFELVERCADQRPESSLLNLISYRAQSIHPAKDGWIQNLQALMERFFRSESRGAVRIKVLDVLSFVLLINRQFYEEELINSVVISQLSHIPEDKDHQVRKLATQLLVDLAEGCHTHHFNSLLDIIEKVMARSLSPPPELEERDVAAYSASLEDVKTAVLGLLVILQTKLYTLPASHATRVYEMLVSHIQLHYKHSYTLPIASSIRLQAFDFLLLLRADSLHRLGLPNKDGVVRFSPYCVCDYMEPERGSEKKTSGPLSPPTGPPGPAPAGPAVRLGSVPYSLLFRVLLQCLKQESDWKVLKLVLGRLPESLRYKVLIFTSPCSVDQLCSALCSMLSGPKTLERLRGAPEGFSRTDLHLAVVPVLTALISYHNYLDKTKQREMVYCLEQGLIHRCASQCVVALSICSVEMPDIIIKALPVLVVKLTHISATASMAVPLLEFLSTLARLPHLYRNFAAEQYASVFAISLPYTNPSKFNQYIVCLAHHVIAMWFIRCRLPFRKDFVPFITKGLRSNVLLSFDDTPEKDSFRARSTSLNERPKSLRIARPPKQGLNNSPPVKEFKESSAAEAFRCRSISVSEHVVRSRIQTSLTSASLGSADENSVAQADDSLKNLHLELTETCLDMMARYVFSNFTAVPKRSPVGEFLLAGGRTKTWLVGNKLVTVTTSVGTGTRSLLGLDSGELQSGPESSSSPGVHVRQTKEAPAKLESQAGQQVSRGARDRVRSMSGGHGLRVGALDVPASQFLGSATSPGPRTAPAAKPEKASAGTRVPVQEKTNLAAYVPLLTQGWAEILVRRPTGNTSWLMSLENPLSPFSSDINNMPLQELSNALMAAERFKEHRDTALYKSLSVPAASTAKPPPLPRSNTVASFSSLYQSSCQGQLHRSVSWADSAVVMEEGSPGEVPVLVEPPGLEDVEAALGMDRRTDAYSRSSSVSSQEEKSLHAEELVGRGIPIERVVSSEGGRPSVDLSFQPSQPLSKSSSSPELQTLQDILGDPGDKADVGRLSPEVKARSQSGTLDGESAAWSASGEDSRGQPEGPLPSSSPRSPSGLRPRGYTISDSAPSRRGKRVERDALKSRATASNAEKVPGINPSFVFLQLYHSPFFGDESNKPILLPNESQSFERSVQLLDQIPSYDTHKIAVLYVGEGQSNSELAILSNEHGSYRYTEFLTGLGRLIELKDCQPDKVYLGGLDVCGEDGQFTYCWHDDIMQAVFHIATLMPTKDVDKHRCDKKRHLGNDFVSIVYNDSGEDFKLGTIKGQFNFVHVIVTPLDYECNLVSLQCRKDMEGLVDTSVAKIVSDRNLPFVARQMALHANMASQVHHSRSNPTDIYPSKWIARLRHIKRLRQRICEEAAYSNPSLPLVHPPSHSKAPAQTPAEPTPGYEVGQRKRLISSVEDFTEFV

SEQ ID NO: 6 - protein, 1814 aa, Mus musculus
MAKPTSKDSGLKEKFKILLGLGTSRPNPRCAEGKQTEFIITSEILRELSGECGLNNRIRMIGQICDVAKTKKLEEHAVEALWKAVSDLLQPERPPEARHAVLTLLKAIVQGQGDRLGVLRALFFKVIKDYPSNEDLHERLEVFKALTDNGRHITYLEEELAEFVLQWMDVGLSSEFLLVLVNLVKFNSCYLDEYIASMVHMICLLCIRTVSSVDIEVSLQVLDAVVCYNCLPAESLPLFIITLCRTINVKELCEPCWKLMRNLLGTHLGHSAIYNMCRIMEDRSYMEDAPLLRGAVFFVGMALWGAHRLYSLKNSPTSVLPSFYEAMTCPNEVVSYEIVLSITRLIKKYRKELQAVTWDILLDIIERLLQQLQNLDSPELKTIVHDLLTTVEELCDQNEFHGSQERYYELVESYADQRPESSLLNLISYRAQSIHPAKDGWIQNLQLLMERFFRNECRSAVAIKVLDVLSFVLLIIRQFYEEELINSVVISQLSHIPEDKDHQVRKLATQLLVDLAEGCHTHHFNSLLDIIEKVMARSLSPPPELEERDLAVHSASLEDVKTAVLGLLVILQTKLYTLPASHATRVYESLISHIQLHYKHGYSLPIASSIRLQAFDFLLLLRADSLHRLGLPNKDGVVRFSPYCLCDCMELDRASEKKASGPLSPPTGPPSPVPMGPAVRLGYLPYSLLFRVLLQCLKQESDWKVLKLVLSRLPESLRYKVLIFTSPCSVDQLSSALCSMLSAPKTLERLRGTPEGFSRTDLHLAVVPVLTALISYHNYLDKTRQREMVYCLEQGLIYRCASQCVVALAICSVEMPDIIIKALPVLVVKLTHISATASMAIPLLEFLSTLARLPHLYRNFVPEQYASVFAISLPYTNPSKFNQYIVCLAHHVIAMWFIRCRLPFRKDFVPYITKGLRSNVLLSFDDTPEKDSFRARSTSLNERPKSLRIARAPKQGLNNSPPVKEFKESCAAEAFRCRSISVSEHVVRSRIQTSLTSASLGSADENSMAQADDNLKNLHLELTETCLDMMARYVFSNFTAVPKRSPVGEFLLAGGRTKTWLVGNKLVTVTTSVGTGTRSLLGLDSGDLQGGSDSSSDPSTHVRQTKEAPAKLESQAGQQVSRGARDRVRSMSGGHGLRVGVLDTSAPYSPGGSASLGPQTAVAAKPEKPPAGAQLPTAEKTNLAAYVPLLTQGWAEILVRRPTGNTSWLMSLENPLSPFSSDINNMPLQELSNALMAAERFKEHGHAPVQVIVSATGCTAKPPTLPRSNTVASFSSLYQPSCQGQLHRSVSWADSAMVLEEGSPGETQVPVEPPELEDFEAALGTDRHCQRPDTYSRSSSASSQEEKSHLEELAAGGIPIERAISSEGARPAVDLSFQPSQPLSKSSSSPELQTLQDILGDLGDKIDIGRLSPEAKVRSQSGILDGEAATWSATGEESRITVPPEGPLPSSSPRSPSGLRPRGYTISDSAPSRRGKRVERDNFKSRAAASSAEKVPGINPSFVFLQLYHSPFFGDESNKPILLPNESFERSVQLLDQIPSYDTHKIAVLYVGEGQSSSELAILSNEHGSYRYTEFLTGLGRLIELKDCQPDKVYLGGLDVCGEDGQFTYCWHDDIMQAVFHIATLMPTKDVDKHRCDKKRHLGNDFVSIIYNDSGEDFKLGTIKQGQFNFVHVIITPLDYKCNLLTLQCRKDGPACKCEWWRQPGEIVVWALPVVMELTVTILLCHLQMASQVHHSRSNPTDIYPSKWIARLRHIKRLRQRIREEVHYSNPSLPLMHPPAHTKAPAQAPEATPTYETGQRKRLISSVDDFTEFV

SEQ ID NO: 7 - protein, 1809 aa, Rattus norvegicus
MAKPTSKDSGLKEKFKILLGLGTSRPNPRCAEGKQTEFIITAEILRELSGECGLNNRIRMIGQICDVAKTKKLEEHAVEALWKAVSDLLQPERPPEARHAVLALLKAIVQGQGDRLGVLRALFFKVIKDYPSNEDLHERLEVFKALTDNGRHITYLEEELAEFVLQWMDVGLSSEFLLVLVNLVKFNSCYLDEYIAPMVHMICLLCIRTVSSVDIEVSLQVLDAVVCYNCLPAESLPLFIITLCRTVNVKELCEPCWKLMRNLLGTHLGHSAIYNMCRIMENRSYMEDAPLLRGAVFFVGMALWGAHRLYSLKNSPTSVLPSFYEAMTCPNEVVSYEIVLSITRLIKKYRKELQAVTWDILLDIIERLLQQLQNLDSPELRTIVHDLLTTVEELCDQNEFHGSQERYYELVESYADQRPESSLLNLITYRAQSIHPAKDGWIQNLQLLMERFFRNECRSAVRIKVLDVLSFVLLINRQFYEEELINSVVISQLSHIPEDKDHQVRKLATQLLVDLAEGCHTHHFNSLLDIIEKVMARSLSPPLELEERDLAVYSASLEDVKTAVLGLLVILQTKLYTLPASHATRVYETLISHIQLHYKHGYSLPIASSIRLQAFDFLLLLRADSLHRLGLPNKDGVVRFSPYCLCDCAELDRASEKKASGPLSPPTGPPSPVPTGPAVRLGHLPYSLLFRVLLQCLKQETDWKVLKLVLSKLPESLRYKVLIFTSPCSVDQLSSALCSMLSAPKTLERLRGTPEGFSRTDLHLAVVPVLTALISYHNYLDKTRQREMVYCLEQGLIYRCASQCVVALAICSVEMPDIIIKALPVLVVKLTHISATASMAIPLLEFLSTLARLPHLYRNFAAEQYASVFAISLPYTNPSKFNQYIVCLAHHVIAMWFIRCRLPFRKDFVPYITKGLRSNVLLSFDDTPEKDKFRARSTSLNERPKSLRIARAPKQGLNNSPPVKEFKESCAAEAFRCRSISVSEHVVRSRIQTSLTSASLGSADENSMAQADDNLKNLHLELTETCLDMMARYVFSNFTAVPKRSPVGEFLLAGGRTKTWLVGNKLVTVTTSVGTGTRSLLGLDSGDLQGGSASSSDPGTHVRQTKEAPAKLESQAGQQVSRGARDRVRSMSGGHGLRVGVLDTSAPYTPGGPASLGAQAAPAARPEKPCAGAQLPAAEKANLAAYVPLLTQGWAEILVRRPTGNTSWLMSLENPLSPFSSDINNMPLQELSNALMAAERFKEHRDTALYKSLSVPAAGTAKPPTLPRSNTVASFSSLYQPSCQGQLHRSVSWADSAVVLEEGSPGEAHVPVEPPELEDFEAALGTDRHCQRPDAYSRSSSASSQEEKSHLEELAAGGIPIERAISSEGARPTVDLSFQPSQPLSKSSSSPELQTLQDILGDLGDKTDIGRLSPEAKVRSQSGILDGEAATWSAPGEESRITVPPEGPLPSSSPRSPSGLRPRGYTISDSAPSRRGKRVERDNFKSRTAASSAEKVPGINPSFVFLQLYHSPFCGDESNKPILLPNESFERSVQLLDQIPSYDTHKIAVLYVGEGQSSSELAILSNEHGSYRYTEFLTGLGRLIELKDCQPDKVYLGGLDVCGEDGQFTYCWHDDIMQAVFHIATLMPTKDVDKHRCDKKRHLGNDFVSIIYNDSGEDFKLGTIKGQFNFVHVIITPLDYKCNLLTLQCRKDMEGLVDTSVAKIVSDRNLSFVARQMALHANMASQVHHRRSNPTDIYPSKWIARLRHIKRLRQRIREEVHYSNPSLPLMHPPAHTKVPAQAPTEATPTYETGQRKRLISSVDDFTEFV

SEQ ID NO: 8 - protein, 1814 aa, Artificial Sequence
  mouse TSC2 polypeptide having a S1365A substitution
MAKPTSKDSGLKEKFKILLGLGTSRPNPRCAEGKQTEFIITSEILRELSGECGLNNRIRMIGQICDVAKTKKLEEHAVEALWKAVSDLLQPERPPEARHAVLTLLKAIVQGQGDRLGVLRALFFKVIKDYPSNEDLHERLEVFKALTDNGRHITYLEEELAEFVLQWMDVGLSSEFLLVLVNLVKFNSCYLDEYIASMVHMICLLCIRTVSSVDIEVSLQVLDAVVCYNCLPAESLPLFIITLCRTINVKELCEPCWKLMRNLLGTHLGHSAIYNMCRIMEDRSYMEDAPLLRGAVFFVGMALWGAHRLYSLKNSPTSVLPSFYEAMTCPNEVVSYEIVLSITRLIKKYRKELQAVTWDILLDIIERLLQQLQNLDSPELKTIVHDLLTTVEELCDQNEFHGSQERYYELVESYADQRPESSLLNLISYRAQSIHPAKDGWIQNLQLLMERFFRNECRSAVAIKVLDVLSFVLLIIRQFYEEELINSVVISQLSHIPEDKDHQVRKLATQLLVDLAEGCHTHHFNSLLDIIEKVMARSLSPPPELEERDLAVHSASLEDVKTAVLGLLVILQTKLYTLPASHATRVYESLISHIQLHYKHGYSLPIASSIRLQAFDFLLLLRADSLHRLGLPNKDGVVRFSPYCLCDCMELDRASEKKASGPLSPPTGPPSPVPMGPAVRLGYLPYSLLFRVLLQCLKQESDWKVLKLVLSRLPESLRYKVLIFTSPCSVDQLSSALCSMLSAPKTLERLRGTPEGFSRTDLHLAVVPVLTALISYHNYLDKTRQREMVYCLEQGLIYRCASQCVVALAICSVEMPDIIIKALPVLVVKLTHISATASMAIPLLEFLSTLARLPHLYRNFVPEQYASVFAISLPYTNPSKFNQYIVCLAHHVIAMWFIRCRLPFRKDFVPYITKGLRSNVLLSFDDTPEKDSFRARSTSLNERPKSLRIARAPKQGLNNSPPVKEFKESCAAEAFRCRSISVSEHVVRSRIQTSLTSASLGSADENSMAQADDNLKNLHLELTETCLDMMARYVFSNFTAVPKRSPVGEFLLAGGRTKTWLVGNKLVTVTTSVGTGTRSLLGLDSGDLQGGSDSSSDPSTHVRQTKEAPAKLESQAGQQVSRGARDRVRSMSGGHGLRVGVLDTSAPYSPGGSASLGPQTAVAAKPEKPPAGAQLPTAEKTNLAAYVPLLTQGWAEILVRRPTGNTSWLMSLENPLSPFSSDINNMPLQELSNALMAAERFKEHGHAPVQVIVSATGCTAKPPTLPRSNTVASFSSLYQPSCQGQLHRSVSWADSAMVLEEGSPGETQVPVEPPELEDFEAALGTDRHCQRPDTYSRSSSASSQEEKSHLEELAAGGIPIERAIASEGARPAVDLSFQPSQPLSKSSSSPELQTLQDILGDLGDKIDIGRLSPEAKVRSQSGILDGEAATWSATGEESRITVPPEGPLPSSSPRSPSGLRPRGYTISDSAPSRRGKRVERDNFKSRAAASSAEKVPGINPSFVFLQLYHSPFFGDESNKPILLPNESFERSVQLLDQIPSYDTHKIAVLYVGEGQSSSELAILSNEHGSYRYTEFLTGLGRLIELKDCQPDKVYLGGLDVCGEDGQFTYCWHDDIMQAVFHIATLMPTKDVDKHRCDKKRHLGNDFVSIIYNDSGEDFKLGTIKQGQFNFVHVIITPLDYKCNLLTLQCRKDGPACKCEWWRQPGEIVVWALPVVMELTVTILLCHLQMASQVHHSRSNPTDIYPSKWIARLRHIKRLRQRIREEVHYSNPSLPLMHPPAHTKAPAQAPEATPTYETGQRKRLISSVDDFTEFV

SEQ ID NO: 9 - protein, 1809 aa, Artificial Sequence
  rat TSC2 polypeptide having a S1366A substitution
MAKPTSKDSGLKEKFKILLGLGTSRPNPRCAEGKQTEFIITAEILRELSGECGLNNRIRMIGQICDVAKTKKLEEHAVEALWKAVSDLLQPERPPEARHAVLALLKAIVQGQGDRLGVLRALFFKVIKDYPSNEDLHERLEVFKALTDNGRHITYLEEELAEFVLQWMDVGLSSEFLLVLVNLVKFNSCYLDEYIAPMVHMICLLCIRTVSSVDIEVSLQVLDAVVCYNCLPAESLPLFIITLCRTVNVKELCEPCWKLMRNLLGTHLGHSAIYNMCRIMENRSYMEDAPLLRGAVFFVGMALWGAHRLYSLKNSPTSVLPSFYEAMTCPNEVVSYEIVLSITRLIKKYRKELQAVTWDILLDIIERLLQQLQNLDSPELRTIVHDLLTTVEELCDQNEFHGSQERYYELVESYADQRPESSLLNLITYRAQSIHPAKDGWIQNLQLLMERFFRNECRSAVRIKVLDVLSFVLLINRQFYEEELINSVVISQLSHIPEDKDHQVRKLATQLLVDLAEGCHTHHFNSLLDIIEKVMARSLSPPLELEERDLAVYSASLEDVKTAVLGLLVILQTKLYTLPASHATRVYETLISHIQLHYKHGYSLPIASSIRLQAFDFLLLLRADSLHRLGLPNKDGVVRFSPYCLCDCAELDRASEKKASGPLSPPTGPPSPVPTGPAVRLGHLPYSLLFRVLLQCLKQETDWKVLKLVLSKLPESLRYKVLIFTSPCSVDQLSSALCSMLSAPKTLERLRGTPEGFSRTDLHLAVVPVLTALISYHNYLDKTRQREMVYCLEQGLIYRCASQCVVALAICSVEMPDIIIKALPVLVVKLTHISATASMAIPLLEFLSTLARLPHLYRNFAAEQYASVFAISLPYTNPSKFNQYIVCLAHHVIAMWFIRCRLPFRKDFVPYITKGLRSNVLLSFDDTPEKDKFRARSTSLNERPKSLRIARAPKQGLNNSPPVKEFKESCAAEAFRCRSISVSEHVVRSRIQTSLTSASLGSADENSMAQADDNLKNLHLELTETCLDMMARYVFSNFTAVPKRSPVGEFLLAGGRTKTWLVGNKLVTVTTSVGTGTRSLLGLDSGDLQGGSASSSDPGTHVRQTKEAPAKLESQAGQQVSRGARDRVRSMSGGHGLRVGVLDTSAPYTPGGPASLGAQAAPAARPEKPCAGAQLPAAEKANLAAYVPLLTQGWAEILVRRPTGNTSWLMSLENPLSPFSSDINNMPLQELSNALMAAERFKEHRDTALYKSLSVPAAGTAKPPTLPRSNTVASFSSLYQPSCQGQLHRSVSWADSAVVLEEGSPGEAHVPVEPPELEDFEAALGTDRHCQRPDAYSRSSSASSQEEKSHLEELAAGGIPIERAIASEGARPTVDLSFQPSQPLSKSSSSPELQTLQDILGDLGDKTDIGRLSPEAKVRSQSGILDGEAATWSAPGEESRITVPPEGPLPSSSPRSPSGLRPRGYTISDSAPSRRGKRVERDNFKSRTAASSAEKVPGINPSFVFLQLYHSPFCGDESNKPILLPNESFERSVQLLDQIPSYDTHKIAVLYVGEGQSSSELAILSNEHGSYRYTEFLTGLGRLIELKDCQPDKVYLGGLDVCGEDGQFTYCWHDDIMQAVFHIATLMPTKDVDKHRCDKKRHLGNDFVSIIYNDSGEDFKLGTIKGQFNFVHVIITPLDYKCNLLTLQCRKDMEGLVDTSVAKIVSDRNLSFVARQMALHANMASQVHHRRSNPTDIYPSKWIARLRHIKRLRQRIREEVHYSNPSLPLMHPPAHTKVPAQAPTEATPTYETGQRKRLISSVDDFTEFV

SEQ ID NO: 10 - protein, 1814 aa, Artificial Sequence
  mouse TSC2 polypeptide having a S1364E substitution
MAKPTSKDSGLKEKFKILLGLGTSRPNPRCAEGKQTEFIITSEILRELSGECGLNNRIRMIGQICDVAKTKKLEEHAVEALWKAVSDLLQPERPPEARHAVLTLLKAIVQGQGDRLGVLRALFFKVIKDYPSNEDLHERLEVFKALTDNGRHITYLEEELAEFVLQWMDVGLSSEFLLVLVNLVKFNSCYLDEYIASMVHMICLLCIRTVSSVDIEVSLQVLDAVVCYNCLPAESLPLFIITLCRTINVKELCEPCWKLMRNLLGTHLGHSAIYNMCRIMEDRSYMEDAPLLRGAVFFVGMALWGAHRLYSLKNSPTSVLPSFYEAMTCPNEVVSYEIVLSITRLIKKYRKELQAVTWDILLDIIERLLQQLQNLDSPELKTIVHDLLTTVEELCDQNEFHGSQERYYELVESYADQRPESSLLNLISYRAQSIHPAKDGWIQNLQLLMERFFRNECRSAVAIKVLDVLSFVLLIIRQFYEEELINSVVISQLSHIPEDKDHQVRKLATQLLVDLAEGCHTHHFNSLLDIIEKVMARSLSPPPELEERDLAVHSASLEDVKTAVLGLLVILQTKLYTLPASHATRVYESLISHIQLHYKHGYSLPIASSIRLQAFDFLLLLRADSLHRLGLPNKDGVVRFSPYCLCDCMELDRASEKKASGPLSPPTGPPSPVPMGPAVRLGYLPYSLLFRVLLQCLKQESDWKVLKLVLSRLPESLRYKVLIFTSPCSVDQLSSALCSMLSAPKTLERLRGTPEGFSRTDLHLAVVPVLTALISYHNYLDKTRQREMVYCLEQGLIYRCASQCVVALAICSVEMPDIIIKALPVLVVKLTHISATASMAIPLLEFLSTLARLPHLYRNFVPEQYASVFAISLPYTNPSKFNQYIVCLAHHVIAMWFIRCRLPFRKDFVPYITKGLRSNVLLSFDDTPEKDSFRARSTSLNERPKSLRIARAPKQGLNNSPPVKEFKESCAAEAFRCRSISVSEHVVRSRIQTSLTSASLGSADENSMAQADDNLKNLHLELTETCLDMMARYVFSNFTAVPKRSPVGEFLLAGGRTKTWLVGNKLVTVTTSVGTGTRSLLGLDSGDLQGGSDSSSDPSTHVRQTKEAPAKLESQAGQQVSRGARDRVRSMSGGHGLRVGVLDTSAPYSPGGSASLGPQTAVAAKPEKPPAGAQLPTAEKTNLAAYVPLLTQGWAEILVRRPTGNTSWLMSLENPLSPFSSDINNMPLQELSNALMAAERFKEHGHAPVQVIVSATGCTAKPPTLPRSNTVASFSSLYQPSCQGQLHRSVSWADSAMVLEEGSPGETQVPVEPPELEDFEAALGTDRHCQRPDTYSRSSSASSQEEKSHLEELAAGGIPIERAIESEGARPAVDLSFQPSQPLSKSSSSPELQTLQDILGDLGDKIDIGRLSPEAKVRSQSGILDGEAATWSATGEESRITVPPEGPLPSSSPRSPSGLRPRGYTISDSAPSRRGKRVERDNFKSRAAASSAEKVPGINPSFVFLQLYHSPFFGDESNKPILLPNESFERSVQLLDQIPSYDTHKIAVLYVGEGQSSSELAILSNEHGSYRYTEFLTGLGRLIELKDCQPDKVYLGGLDVCGEDGQFTYCWHDDIMQAVFHIATLMPTKDVDKHRCDKKRHLGNDFVSIIYNDSGEDFKLGTIKQGQFNFVHVIITPLDYKCNLLTLQCRKDGPACKCEWWRQPGEIVVWALPVVMELTVTILLCHLQMASQVHHSRSNPTDIYPSKWIARLRHIKRLRQRIREEVHYSNPSLPLMHPPAHTKAPAQAPEATPTYETGQRKRLISSVDDFTEFV

SEQ ID NO: 11 - protein, 1809 aa, Artificial Sequence
  rat TSC2 polypeptide having a S1364E substitution
MAKPTSKDSGLKEKFKILLGLGTSRPNPRCAEGKQTEFIITAEILRELSGECGLNNRIRMIGQICDVAKTKKLEEHAVEALWKAVSDLLQPERPPEARHAVLALLKAIVQGQGDRLGVLRALFFKVIKDYPSNEDLHERLEVFKALTDNGRHITYLEEELAEFVLQWMDVGLSSEFLLVLVNLVKFNSCYLDEYIAPMVHMICLLCIRTVSSVDIEVSLQVLDAVVCYNCLPAESLPLFIITLCRTVNVKELCEPCWKLMRNLLGTHLGHSAIYNMCRIMENRSYMEDAPLLRGAVFFVGMALWGAHRLYSLKNSPTSVLPSFYEAMTCPNEVVSYEIVLSITRLIKKYRKELQAVTWDILLDIIERLLQQLQNLDSPELRTIVHDLLTTVEELCDQNEFHGSQERYYELVESYADQRPESSLLNLITYRAQSIHPAKDGWIQNLQLLMERFFRNECRSAVRIKVLDVLSFVLLINRQFYEEELINSVVISQLSHIPEDKDHQVRKLATQLLVDLAEGCHTHHFNSLLDIIEKVMARSLSPPLELEERDLAVYSASLEDVKTAVLGLLVILQTKLYTLPASHATRVYETLISHIQLHYKHGYSLPIASSIRLQAFDFLLLLRADSLHRLGLPNKDGVVRFSPYCLCDCAELDRASEKKASGPLSPPTGPPSPVPTGPAVRLGHLPYSLLFRVLLQCLKQETDWKVLKLVLSKLPESLRYKVLIFTSPCSVDQLSSALCSMLSAPKTLERLRGTPEGFSRTDLHLAVVPVLTALISYHNYLDKTRQREMVYCLEQGLIYRCASQCVVALAICSVEMPDIIIKALPVLVVKLTHISATASMAIPLLEFLSTLARLPHLYRNFAAEQYASVFAISLPYTNPSKFNQYIVCLAHHVIAMWFIRCRLPFRKDFVPYITKGLRSNVLLSFDDTPEKDKFRARSTSLNERPKSLRIARAPKQGLNNSPPVKEFKESCAAEAFRCRSISVSEHVVRSRIQTSLTSASLGSADENSMAQADDNLKNLHLELTETCLDMMARYVFSNFTAVPKRSPVGEFLLAGGRTKTWLVGNKLVTVTTSVGTGTRSLLGLDSGDLQGGSASSSDPGTHVRQTKEAPAKLESQAGQQVSRGARDRVRSMSGGHGLRVGVLDTSAPYTPGGPASLGAQAAPAARPEKPCAGAQLPAAEKANLAAYVPLLTQGWAEILVRRPTGNTSWLMSLENPLSPFSSDINNMPLQELSNALMAAERFKEHRDTALYKSLSVPAAGTAKPPTLPRSNTVASFSSLYQPSCQGQLHRSVSWADSAVVLEEGSPGEAHVPVEPPELEDFEAALGTDRHCQRPDAYSRSSSASSQEEKSHLEELAAGGIPIERAIESEGARPTVDLSFQPSQPLSKSSSSPELQTLQDILGDLGDKTDIGRLSPEAKVRSQSGILDGEAATWSAPGEESRITVPPEGPLPSSSPRSPSGLRPRGYTISDSAPSRRGKRVERDNFKSRTAASSAEKVPGINPSFVFLQLYHSPFCGDESNKPILLPNESFERSVQLLDQIPSYDTHKIAVLYVGEGQSSSELAILSNEHGSYRYTEFLTGLGRLIELKDCQPDKVYLGGLDVCGEDGQFTYCWHDDIMQAVFHIATLMPTKDVDKHRCDKKRHLGNDFVSIIYNDSGEDFKLGTIKGQFNFVHVIITPLDYKCNLLTLQCRKDMEGLVDTSVAKIVSDRNLSFVARQMALHANMASQVHHRRSNPTDIYPSKWIARLRHIKRLRQRIREEVHYSNPSLPLMHPPAHTKVPAQAPTEATPTYETGQRKRLISSVDDFTEFV